European Patent Specification EP 3 813 531 B1, published February 21, 2024. Title: PEPTIDE ANALOGS OF NATURAL PEPTAIBOL TRICHOGIN GA IV WITH PHYTOSANITARY ACTIVITY. Applicant: UNIVERSITA' DEGLI STUDI DI PADOVA. The sequence listing filed with the application follows.

SEQUENCE LISTING (9 sequences)

SEQ ID NO: 1 - protein, 11 aa, Artificial Sequence
  NON_STD 1: 1 octanoil Aib
  PEP4
  NON_STD 4: Aib
  NON_STD 5: Lys(HCl)
  NON_STD 6: Lys(HCl)
  NON_STD 8: Aib
  NON_STD 11: Lol
XGLXXXLXGIX

SEQ ID NO: 2 - protein, 11 aa, Artificial Sequence
  NON_STD 1: 1 ottanoile Aib
  PEP4-rink
  NON_STD 4: Aib
  NON_STD 5: Lys(HCl)
  NON_STD 6: Lys(HCl)
  NON_STD 8: Aib
XGLXXXLXGIL

SEQ ID NO: 3 - protein, 11 aa, Artificial Sequence
  NON_STD 1: 1 ottanoile Aib
  K6-Lol
  NON_STD 4: Aib
  NON_STD 6: Lys(HCl)
  NON_STD 8: Aib
  NON_STD 11: Lol
XGLXGXLXGIX

SEQ ID NO: 4 - protein, 11 aa, Artificial Sequence
  NON_STD 1: 1 ottanoile Aib
  K6-rink
  NON_STD 4: Aib
  NON_STD 6: Lys(HCl)
  NON_STD 8: Aib
XGLXGXLXGIL

SEQ ID NO: 5 - protein, 8 aa, Artificial Sequence
  NON_STD 1: 1 ottanoile Aib
  PEP4-corto
  NON_STD 4: Aib
  NON_STD 5: Lys(HCl)
  NON_STD 6: Lys(HCl)
  NON_STD 8: Lol
XGLXXXLX

SEQ ID NO: 6 - protein, 8 aa, Artificial Sequence
  NON_STD 1: 1 ottanoile Aib
  PEP4-corto1-rink
  NON_STD 4: Aib
  NON_STD 5: Lys(HCl)
  NON_STD 6: Lys(HCl)
XGLXXXLL

SEQ ID NO: 7 - protein, 8 aa, Artificial Sequence
  NON_STD 1: 1 ottanoile Aib
  PEP4-corto2-rink
  NON_STD 2: Lys(HCl)
  NON_STD 3: Lys(HCl)
  NON_STD 5: Aib
XXXLXGIL

SEQ ID NO: 8 - protein, 11 aa, Artificial Sequence
  NON_STD 1: 1 ottanoile Aib
  K25
  NON_STD 2: Lys(HCl)
  NON_STD 4: Aib
  NON_STD 5: Lys(HCl)
  NON_STD 8: Aib
  NON_STD 11: Lol
XXLXXGLXGIX

SEQ ID NO: 9 - protein, 11 aa, Artificial Sequence
  NON_STD 1: 1 ottanoile Aib
  peptide tricogina GA IV
  NON_STD 4: Aib
  NON_STD 8: Aib
  NON_TER 11: Lol
XGLXGGLXGIX